European Patent Specification EP 3 500 592 B1, published May 29, 2024. Title: PEPTIDES WITH VASODILATORY AND/OR DIURETIC FUNCTIONS. Applicant: National University of Singapore. The sequence listing filed with the application follows.

SEQUENCE LISTING (56 sequences)

SEQ ID NO: 1 - protein, 17 aa, Artificial Sequence
  K-ring derived 17 aa peptide #1
  MISC_FEATURE (3)..(4): Xaa comprises any amino acid
  MISC_FEATURE (5)..(5): Xaa comprises R or K
  MISC_FEATURE (6)..(6): Xaa comprises M, I or L
  MISC_FEATURE (10)..(10): Xaa comprises G, S or N
  MISC_FEATURE (11)..(11): Xaa comprises A, H or S
  MISC_FEATURE (12)..(12): Xaa comprises Q, T, S, M or V
  MISC_FEATURE (14)..(14): Xaa comprises any amino acid
  MISC_FEATURE (15)..(15): Xaa comprises I or L
CFXXXXDRIXXXSXXGC

SEQ ID NO: 2 - protein, 17 aa, Artificial Sequence
  K-ring derived 17 aa peptide #2
  MISC_FEATURE (3)..(3): Xaa comprises D or G
  MISC_FEATURE (4)..(4): Xaa comprises any amino acid
  MISC_FEATURE (5)..(5): Xaa comprises R or K
  MISC_FEATURE (6)..(6): Xaa comprises M, I or L
  MISC_FEATURE (10)..(10): Xaa comprises G, S or N
  MISC_FEATURE (11)..(11): Xaa comprises A, H or S
  MISC_FEATURE (12)..(12): Xaa comprises Q, T, S, M or V
  MISC_FEATURE (14)..(14): Xaa comprises any amino acid
  MISC_FEATURE (15)..(15): Xaa comprises I or L
CFXXXXDRIXXXSXXGC

SEQ ID NO: 3 - protein, 17 aa, Artificial Sequence
  K-ring derived 17 aa peptide #3
  MISC_FEATURE (3)..(3): Xaa comprises any amino acid
  MISC_FEATURE (4)..(4): Xaa comprises R or G
  MISC_FEATURE (5)..(5): Xaa comprises R or K
  MISC_FEATURE (6)..(6): Xaa comprises M, I or L
  MISC_FEATURE (10)..(10): Xaa comprises G, S or N
  MISC_FEATURE (11)..(11): Xaa comprises A, H or S
  MISC_FEATURE (12)..(12): Xaa comprises Q, T, S, M or V
  MISC_FEATURE (14)..(14): Xaa comprises any amino acid
  MISC_FEATURE (15)..(15): Xaa comprises I or L
CFXXXXDRIXXXSXXGC

SEQ ID NO: 4 - protein, 17 aa, Artificial Sequence
  K-ring derived 17 aa peptide #4
  MISC_FEATURE (3)..(4): Xaa comprises any amino acid
  MISC_FEATURE (5)..(5): Xaa comprises R or K
  MISC_FEATURE (6)..(6): Xaa comprises M, I or L
  MISC_FEATURE (10)..(10): Xaa comprises G, S or N
  MISC_FEATURE (11)..(11): Xaa comprises A, H or S
  MISC_FEATURE (12)..(12): Xaa comprises Q, T, S, M or V
  MISC_FEATURE (14)..(14): Xaa comprises D or G
  MISC_FEATURE (15)..(15): Xaa comprises I or L
CFXXXXDRIXXXSXXGC

SEQ ID NO: 5 - protein, 17 aa, Artificial Sequence
  K-ring derived 17 aa peptide #5
  MISC_FEATURE (4)..(4): Xaa comprises any amino acid
  MISC_FEATURE (5)..(5): Xaa comprises R or K
  MISC_FEATURE (6)..(6): Xaa comprises M, I or L
  MISC_FEATURE (10)..(10): Xaa comprises G, S or N
  MISC_FEATURE (11)..(11): Xaa comprises A, H or S
  MISC_FEATURE (12)..(12): Xaa comprises Q, T, S, M or V
  MISC_FEATURE (14)..(14): Xaa comprises any amino acid
  MISC_FEATURE (15)..(15): Xaa comprises I or L
CFDXXXDRIXXXSXXGC

SEQ ID NO: 6 - protein, 17 aa, Artificial Sequence
  K-ring derived 17 aa peptide #6
  MISC_FEATURE (4)..(4): Xaa comprises any amino acid
  MISC_FEATURE (5)..(5): Xaa comprises R or K
  MISC_FEATURE (6)..(6): Xaa comprises M, I or L
  MISC_FEATURE (10)..(10): Xaa comprises G, S or N
  MISC_FEATURE (11)..(11): Xaa comprises A, H or S
  MISC_FEATURE (12)..(12): Xaa comprises Q, T, S, M or V
  MISC_FEATURE (14)..(14): Xaa comprises any amino acid
  MISC_FEATURE (15)..(15): Xaa comprises I or L
CFGXXXDRIXXXSXXGC

SEQ ID NO: 7 - protein, 17 aa, Artificial Sequence
  K-ring derived 17 aa peptide #7
  MISC_FEATURE (3)..(3): Xaa comprises any amino acid
  MISC_FEATURE (5)..(5): Xaa comprises R or K
  MISC_FEATURE (6)..(6): Xaa comprises M, I or L
  MISC_FEATURE (10)..(10): Xaa comprises G, S or N
  MISC_FEATURE (11)..(11): Xaa comprises A, H or S
  MISC_FEATURE (12)..(12): Xaa comprises Q, T, S, M or V
  MISC_FEATURE (14)..(14): Xaa comprises any amino acid
  MISC_FEATURE (15)..(15): Xaa comprises I or L
CFXRXXDRIXXXSXXGC

SEQ ID NO: 8 - protein, 17 aa, Artificial Sequence
  K-ring derived 17 aa peptide #8
  MISC_FEATURE (3)..(3): Xaa comprises any amino acid
  MISC_FEATURE (5)..(5): Xaa comprises R or K
  MISC_FEATURE (6)..(6): Xaa comprises M, I or L
  MISC_FEATURE (10)..(10): Xaa comprises G, S or N
  MISC_FEATURE (11)..(11): Xaa comprises A, H or S
  MISC_FEATURE (12)..(12): Xaa comprises Q, T, S, M or V
  MISC_FEATURE (14)..(14): Xaa comprises any amino acid
  MISC_FEATURE (15)..(15): Xaa comprises I or L
CFXGXXDRIXXXSXXGC

SEQ ID NO: 9 - protein, 17 aa, Artificial Sequence
  K-ring derived 17 aa peptide #9
  MISC_FEATURE (3)..(4): Xaa comprises any amino acid
  MISC_FEATURE (5)..(5): Xaa comprises R or K
  MISC_FEATURE (6)..(6): Xaa comprises M, I or L
  MISC_FEATURE (10)..(10): Xaa comprises G, S or N
  MISC_FEATURE (11)..(11): Xaa comprises A, H or S
  MISC_FEATURE (12)..(12): Xaa comprises Q, T, S, M or V
  MISC_FEATURE (15)..(15): Xaa comprises I or L
CFXXXXDRIXXXSDXGC

SEQ ID NO: 10 - protein, 17 aa, Artificial Sequence
  K-ring derived 17 aa peptide #10
  MISC_FEATURE (3)..(4): Xaa comprises any amino acid
  MISC_FEATURE (5)..(5): Xaa comprises R or K
  MISC_FEATURE (6)..(6): Xaa comprises M, I or L
  MISC_FEATURE (10)..(10): Xaa comprises G, S or N
  MISC_FEATURE (11)..(11): Xaa comprises A, H or S
  MISC_FEATURE (12)..(12): Xaa comprises Q, T, S, M or V
  MISC_FEATURE (15)..(15): Xaa comprises I or L
CFXXXXDRIXXXSGXGC

SEQ ID NO: 11 - protein, 17 aa, Artificial Sequence
  K-ring derived 17 aa peptide #11
  MISC_FEATURE (5)..(5): Xaa comprises R or K
  MISC_FEATURE (6)..(6): Xaa comprises M, I or L
  MISC_FEATURE (10)..(10): Xaa comprises G, S or N
  MISC_FEATURE (11)..(11): Xaa comprises A, H or S
  MISC_FEATURE (12)..(12): Xaa comprises Q, T, S, M or V
  MISC_FEATURE (14)..(14): Xaa comprises any amino acid
  MISC_FEATURE (15)..(15): Xaa comprises I or L
CFDRXXDRIXXXSXXGC

SEQ ID NO: 12 - protein, 17 aa, Artificial Sequence
  K-ring derived 17 aa peptide #12
  MISC_FEATURE (5)..(5): Xaa comprises R or K
  MISC_FEATURE (6)..(6): Xaa comprises M, I or L
  MISC_FEATURE (10)..(10): Xaa comprises G, S or N
  MISC_FEATURE (11)..(11): Xaa comprises A, H or S
  MISC_FEATURE (12)..(12): Xaa comprises Q, T, S, M or V
  MISC_FEATURE (14)..(14): Xaa comprises any amino acid
  MISC_FEATURE (15)..(15): Xaa comprises I or L
CFGRXXDRIXXXSXXGC

SEQ ID NO: 13 - protein, 17 aa, Artificial Sequence
  K-ring derived 17 aa peptide #13
  MISC_FEATURE (5)..(5): Xaa comprises R or K
  MISC_FEATURE (6)..(6): Xaa comprises M, I or L
  MISC_FEATURE (10)..(10): Xaa comprises G, S or N
  MISC_FEATURE (11)..(11): Xaa comprises A, H or S
  MISC_FEATURE (12)..(12): Xaa comprises Q, T, S, M or V
  MISC_FEATURE (14)..(14): Xaa comprises any amino acid
  MISC_FEATURE (15)..(15): Xaa comprises I or L
CFDGXXDRIXXXSXXGC

SEQ ID NO: 14 - protein, 17 aa, Artificial Sequence
  K-ring derived 17 aa peptide #14
  MISC_FEATURE (5)..(5): Xaa comprises R or K
  MISC_FEATURE (6)..(6): Xaa comprises M, I or L
  MISC_FEATURE (10)..(10): Xaa comprises G, S or N
  MISC_FEATURE (11)..(11): Xaa comprises A, H or S
  MISC_FEATURE (12)..(12): Xaa comprises Q, T, S, M or V
  MISC_FEATURE (14)..(14): Xaa comprises any amino acid
  MISC_FEATURE (15)..(15): Xaa comprises I or L
CFGGXXDRIXXXSXXGC

SEQ ID NO: 15 - protein, 17 aa, Artificial Sequence
  K-ring derived 17 aa peptide #15
  MISC_FEATURE (4)..(4): Xaa comprises any amino acid
  MISC_FEATURE (5)..(5): Xaa comprises R or K
  MISC_FEATURE (6)..(6): Xaa comprises M, I or L
  MISC_FEATURE (10)..(10): Xaa comprises G, S or N
  MISC_FEATURE (11)..(11): Xaa comprises A, H or S
  MISC_FEATURE (12)..(12): Xaa comprises Q, T, S, M or V
  MISC_FEATURE (15)..(15): Xaa comprises I or L
CFDXXXDRIXXXSDXGC

SEQ ID NO: 16 - protein, 17 aa, Artificial Sequence
  K-ring derived 17 aa peptide #16
  MISC_FEATURE (4)..(4): Xaa comprises any amino acid
  MISC_FEATURE (5)..(5): Xaa comprises R or K
  MISC_FEATURE (6)..(6): Xaa comprises M, I or L
  MISC_FEATURE (10)..(10): Xaa comprises G, S or N
  MISC_FEATURE (11)..(11): Xaa comprises A, H or S
  MISC_FEATURE (12)..(12): Xaa comprises Q, T, S, M or V
  MISC_FEATURE (15)..(15): Xaa comprises I or L
CFGXXXDRIXXXSDXGC

SEQ ID NO: 17 - protein, 17 aa, Artificial Sequence
  K-ring derived 17 aa peptide #17
  MISC_FEATURE (4)..(4): Xaa comprises any amino acid
  MISC_FEATURE (5)..(5): Xaa comprises R or K
  MISC_FEATURE (6)..(6): Xaa comprises M, I or L
  MISC_FEATURE (10)..(10): Xaa comprises G, S or N
  MISC_FEATURE (11)..(11): Xaa comprises A, H or S
  MISC_FEATURE (12)..(12): Xaa comprises Q, T, S, M or V
  MISC_FEATURE (15)..(15): Xaa comprises I or L
CFDXXXDRIXXXSGXGC

SEQ ID NO: 18 - protein, 17 aa, Artificial Sequence
  K-ring derived 17 aa peptide #18
  MISC_FEATURE (4)..(4): Xaa comprises any amino acid
  MISC_FEATURE (5)..(5): Xaa comprises R or K
  MISC_FEATURE (6)..(6): Xaa comprises M, I or L
  MISC_FEATURE (10)..(10): Xaa comprises G, S or N
  MISC_FEATURE (11)..(11): Xaa comprises A, H or S
  MISC_FEATURE (12)..(12): Xaa comprises Q, T, S, M or V
  MISC_FEATURE (15)..(15): Xaa comprises I or L
CFGXXXDRIXXXSGXGC

SEQ ID NO: 19 - protein, 17 aa, Artificial Sequence
  K-ring derived 17 aa peptide #19
  MISC_FEATURE (3)..(3): Xaa comprises any amino acid
  MISC_FEATURE (5)..(5): Xaa comprises R or K
  MISC_FEATURE (6)..(6): Xaa comprises M, I or L
  MISC_FEATURE (10)..(10): Xaa comprises G, S or N
  MISC_FEATURE (11)..(11): Xaa comprises A, H or S
  MISC_FEATURE (12)..(12): Xaa comprises Q, T, S, M or V
  MISC_FEATURE (15)..(15): Xaa comprises I or L
CFXRXXDRIXXXSDXGC

SEQ ID NO: 20 - protein, 17 aa, Artificial Sequence
  K-ring derived 17 aa peptide #20
  MISC_FEATURE (3)..(3): Xaa comprises any amino acid
  MISC_FEATURE (5)..(5): Xaa comprises R or K
  MISC_FEATURE (6)..(6): Xaa comprises M, I or L
  MISC_FEATURE (10)..(10): Xaa comprises G, S or N
  MISC_FEATURE (11)..(11): Xaa comprises A, H or S
  MISC_FEATURE (12)..(12): Xaa comprises Q, T, S, M or V
  MISC_FEATURE (15)..(15): Xaa comprises I or L
CFXRXXDRIXXXSGXGC

SEQ ID NO: 21 - protein, 17 aa, Artificial Sequence
  K-ring derived 17 aa peptide #21
  MISC_FEATURE (3)..(3): Xaa comprises any amino acid
  MISC_FEATURE (5)..(5): Xaa comprises R or K
  MISC_FEATURE (6)..(6): Xaa comprises M, I or L
  MISC_FEATURE (10)..(10): Xaa comprises G, S or N
  MISC_FEATURE (11)..(11): Xaa comprises A, H or S
  MISC_FEATURE (12)..(12): Xaa comprises Q, T, S, M or V
  MISC_FEATURE (15)..(15): Xaa comprises I or L
CFXGXXDRIXXXSDXGC

SEQ ID NO: 22 - protein, 17 aa, Artificial Sequence
  K-ring derived 17 aa peptide #22
  MISC_FEATURE (3)..(3): Xaa comprises any amino acid
  MISC_FEATURE (5)..(5): Xaa comprises R or K
  MISC_FEATURE (6)..(6): Xaa comprises M, I or L
  MISC_FEATURE (10)..(10): Xaa comprises G, S or N
  MISC_FEATURE (11)..(11): Xaa comprises A, H or S
  MISC_FEATURE (12)..(12): Xaa comprises Q, T, S, M or V
  MISC_FEATURE (15)..(15): Xaa comprises I or L
CFXGXXDRIXXXSGXGC

SEQ ID NO: 23 - protein, 22 aa, Artificial Sequence
  K-ring derived 22 aa peptide #23
  MISC_FEATURE (3)..(4): Xaa comprises any amino acid
  MISC_FEATURE (5)..(5): Xaa comprises R or K
  MISC_FEATURE (6)..(6): Xaa comprises M, I or L
  MISC_FEATURE (10)..(10): Xaa comprises G, S or N
  MISC_FEATURE (11)..(11): Xaa comprises A, H or S
  MISC_FEATURE (12)..(12): Xaa comprises Q, T, S, M or V
  MISC_FEATURE (14)..(14): Xaa comprises any amino acid
  MISC_FEATURE (15)..(15): Xaa comprises I or L
CFXXXXDRIXXXSXXGCNSFRY

SEQ ID NO: 24 - protein, 17 aa, Artificial Sequence
  K-ring derived 17 aa peptide #24
CFDRRIDRISHTSDIGC

SEQ ID NO: 25 - protein, 17 aa, Artificial Sequence
  K-ring derived 17 aa peptide #25
CFGRRIDRISHTSDIGC

SEQ ID NO: 26 - protein, 17 aa, Artificial Sequence
  K-ring derived 17 aa peptide #26
CFDGRIDRISHTSDIGC

SEQ ID NO: 27 - protein, 17 aa, Artificial Sequence
  K-ring derived 17 aa peptide #27
CFDRRIDRISHTSGIGC

SEQ ID NO: 28 - protein, 17 aa, Artificial Sequence
  K-ring derived 17 aa peptide #28
CFGGRIDRISHTSDIGC

SEQ ID NO: 29 - protein, 17 aa, Artificial Sequence
  K-ring derived 17 aa peptide #29
CFGRRIDRISHTSGIGC

SEQ ID NO: 30 - protein, 17 aa, Artificial Sequence
  K-ring derived 17 aa peptide #30
CFDGRIDRISHTSGIGC

SEQ ID NO: 31 - protein, 17 aa, Artificial Sequence
  K-ring derived 17 aa peptide #31
CFGGRIDRISHTSGIGC

SEQ ID NO: 32 - protein, 24 aa, Artificial Sequence
  KNP derived peptide #1
GLLISCFDRRIDRISHTSDIGCRH

SEQ ID NO: 33 - protein, 24 aa, Artificial Sequence
  KNP derived peptide #2
GLLISCFDRRIDRISHTSGIGCRH

SEQ ID NO: 34 - protein, 24 aa, Artificial Sequence
  KNP derived peptide #3
GLLISCFGRRIDRISHTSDIGCRH

SEQ ID NO: 35 - protein, 24 aa, Artificial Sequence
  KNP derived peptide #4
GLLISCFDGRIDRISHTSDIGCRH

SEQ ID NO: 36 - protein, 24 aa, Artificial Sequence
  KNP derived peptide #5
GLLISCFGRRIDRISHTSGIGCRH

SEQ ID NO: 37 - protein, 27 aa, Artificial Sequence
  KNP derived peptide #6
GLLISCFDRRIDRISHTSDIGCNSFRY

SEQ ID NO: 38 - protein, 60 aa, Artificial Sequence
  KNP derived peptide #7
GLLISCFGRRIDRISHTSDIGCRHRKDPPRAPPAAPSAAPLAVTWLIRDLRADSKQSRAA

SEQ ID NO: 39 - protein, 60 aa, Artificial Sequence
  KNP derived peptide #8
GLLISCFDGRIDRISHTSDIGCRHRKDPPRAPPAAPSAAPLAVTWLIRDLRADSKQSRAA

SEQ ID NO: 40 - protein, 60 aa, Artificial Sequence
  KNP derived peptide #9
GLLISCFDRRIDRISHTSGIGCRHRKDPPRAPPAAPSAAPLAVTWLIRDLRADSKQSRAA

SEQ ID NO: 41 - protein, 60 aa, Artificial Sequence
  KNP derived peptide #10
GLLISCFGGRIDRISHTSDIGCRHRKDPPRAPPAAPSAAPLAVTWLIRDLRADSKQSRAA

SEQ ID NO: 42 - protein, 60 aa, Artificial Sequence
  KNP derived peptide #11
GLLISCFGRRIDRISHTSGIGCRHRKDPPRAPPAAPSAAPLAVTWLIRDLRADSKQSRAA

SEQ ID NO: 43 - protein, 60 aa, Artificial Sequence
  KNP derived peptide #12
GLLISCFDGRIDRISHTSGIGCRHRKDPPRAPPAAPSAAPLAVTWLIRDLRADSKQSRAA

SEQ ID NO: 44 - protein, 60 aa, Artificial Sequence
  KNP derived peptide #13
GLLISCFGGRIDRISHTSGIGCRHRKDPPRAPPAAPSAAPLAVTWLIRDLRADSKQSRAA

SEQ ID NO: 45 - protein, 28 aa, Artificial Sequence
  ANP derived peptide #1
SLRRSSCFDGRMERIGAQSGLGCNSFRY

SEQ ID NO: 46 - protein, 28 aa, Artificial Sequence
  ANP derived peptide #2
SLRRSSCFGRRMDRIGAQSGLGCNSFRY

SEQ ID NO: 47 - protein, 28 aa, Artificial Sequence
  ANP derived peptide #3
SLRRSSCFGGRMDRIGAQSDLGCNSFRY

SEQ ID NO: 48 - protein, 28 aa, Artificial Sequence
  ANP derived peptide #4
SLRRSSCFDRRMDRIGAQSGLGCNSFRY

SEQ ID NO: 49 - protein, 28 aa, Artificial Sequence
  ANP derived peptide #5
SLRRSSCFDGRMDRIGAQSDLGCNSFRY

SEQ ID NO: 50 - protein, 28 aa, Artificial Sequence
  ANP derived peptide #6
SLRRSSCFGRRMDRIGAQSDLGCNSFRY

SEQ ID NO: 51 - protein, 28 aa, Artificial Sequence
  ANP derived peptide #7
SLRRSSCFDRRMDRIGAQSDLGCNSFRY

SEQ ID NO: 52 - protein, 28 aa, Homo sapiens
SLRRSSCFGGRMDRIGAQSGLGCNSFRY

SEQ ID NO: 53 - protein, 60 aa, Bungarus caeruleus
GLLISCFDRRIDRISHTSDIGCRHRKDPPRAPPAAPSAAPLAVTWLIRDLRADSKQSRAA

SEQ ID NO: 54 - protein, 32 aa, Homo sapiens
SPKMVQGSGCFGRKMDRISSSSGLGCKVLRRH

SEQ ID NO: 55 - protein, 22 aa, Homo sapiens
GLSKGCFGLKLDRIGSMSGLGC

SEQ ID NO: 56 - protein, 38 aa, Dendroaspis angusticeps
EVKYDPCFGHKIDRINHVSNLGCPSLRDPRPNAPSTSA